European Patent Specification EP 3 883 932 B1, published March 29, 2023. Title: Inhibitors of Gli1 as Therapeutic Agents. Applicant: New York University. The sequence listing filed with the application follows.

SEQUENCE LISTING (5 sequences)

SEQ ID NO: 1 - DNA, 21 bp, Artificial Sequence
  Gli 1 inhibitor siRNA
gucauuaucaaauuucucctt

SEQ ID NO: 2 - DNA, 21 bp, Artificial Sequence
  Gli 1 inhibitor siRNA
agaagaaaagagugggccctt

SEQ ID NO: 3 - DNA, 21 bp, Artificial Sequence
  Gli 1 inhibitor siRNA
uccgguguuuucuucaucctt

SEQ ID NO: 4 - DNA, 21 bp, Artificial Sequence
  Gli1 inhibitor siRNA
gagaucuucccuucauacctt

SEQ ID NO: 5 - DNA, 21 bp, Artificial Sequence
  Gli 1 inhibitor siRNA
aacuccacaggcauacaggau